European Patent Application EP 4 685 236 A1, published January 28, 2026. Title: Temperature sensitive minus strand RNA viruses or virus vectors, and RNA genome thereof. Applicant: Repli-tech Co., Ltd. The sequence listing filed with the application follows.

SEQUENCE LISTING (33 sequences)

SEQ ID NO: 1 - protein, 568 aa, Sendai virus
MDQDAFILKEDSEVEREAPGGRESLSDVIGFLDAVLSSEPTDIGGDRSWLHNTINTPQGPGSAHRAKSEGEGEVSTPSTQDNRSGEESRVSGRTSKPEAEAHAGNLDKQNIHRAFGGRTGTNSVSQDLGDGGDSGILENPPNERGYPRSGIEDENREMAAHPDKRGEDQAEGLPEEVRGSTSLPDEGEGGASNNGRSMEPGSSHSARVTGVLVIPSPELEEAVLRRNKRRPTNSGSKPLTPATVPGTRSPPLNRYNSTGSPPGKPPSTQDEHINSGDTPAVRVKDRKPPIGTRSVSDCPANGRPIHPGLETDSTKKGIGENTSSMKEMATLLTSLGVIQSAQEFESSRDASYVFARRALKSANYAEMTFNVCGLILSAEKSSARKVDENKQLLKQIQESVESFRDIYKRFSEYQKEQNSLLMSNLSTLHIITDRGGKTDNTDSLTRSPSVFAKSKENKTKATRFDPSMETLEDMKYKPDLIREDEFRDEIRNPVYQERDTEPRASNASRLLPSKEKPTMHSLRLVIESSPLSRAEKVAYVKSLSKCKTDQEVKAVMELVEEDIESLTN

SEQ ID NO: 2 - protein, 568 aa, synthetic construct
  REGION 1..568: note = Sendai virus Protein mutant P2
MDQDAFILKEDSEVEREAPGGRESLSDVIGFLDAVLSSEPTDIGGDRSWLHNTINTPQGPGSAHRAKSEGEGEVSTPSTQDNRSGEESRVSGRTSKPEAEAHAGNLDKQNIHRAFGGRTGTNSVSQDLGDGGDSGILENPPNERGYPRSGIEDENREMAAHPDKRGEDQAEGLPEEVRGSTSLPDEGEGGASNNGRSMEPGSSHSARVTGVLVIPSPELEEAVLRRNKRRPTNSGSKPLTPATVPGTRSPPLNRYNSTGSPPGKPPSTQDEHINSGDTPAVRVKDRKPPIGTRSVSDCPANGRPIHPGLETDSTKKGIGENTSSMKEMATLLTSLGVIQSAQEFESSRDASYVFARRALKSANYAEMTFNVCGLILSAEKSSARKVDENKQLLKQIQESVESFRDIYKRFSEYQKEQNSLLMSNLSTLHIITAAGGATDNTDSLTRSPSVFAKSKENKTKATRFDPSMETLEDMKYKPDLIREDEFRDEIRNPVYQERDTEPRASNASRLFPSKEKPTMHSLRLVIESSPLSRAEKVAYVKSLSKCKTDQEVKAVMELVEEDIESLTN

SEQ ID NO: 3 - protein, 568 aa, synthetic construct
  REGION 1..568: note = Sendai virus P protein L511F mutant
MDQDAFILKEDSEVEREAPGGRESLSDVIGFLDAVLSSEPTDIGGDRSWLHNTINTPQGPGSAHRAKSEGEGEVSTPSTQDNRSGEESRVSGRTSKPEAEAHAGNLDKQNIHRAFGGRTGTNSVSQDLGDGGDSGILENPPNERGYPRSGIEDENREMAAHPDKRGEDQAEGLPEEVRGSTSLPDEGEGGASNNGRSMEPGSSHSARVTGVLVIPSPELEEAVLRRNKRRPTNSGSKPLTPATVPGTRSPPLNRYNSTGSPPGKPPSTQDEHINSGDTPAVRVKDRKPPIGTRSVSDCPANGRPIHPGLETDSTKKGIGENTSSMKEMATLLTSLGVIQSAQEFESSRDASYVFARRALKSANYAEMTFNVCGLILSAEKSSARKVDENKQLLKQIQESVESFRDIYKRFSEYQKEQNSLLMSNLSTLHIITDRGGKTDNTDSLTRSPSVFAKSKENKTKATRFDPSMETLEDMKYKPDLIREDEFRDEIRNPVYQERDTEPRASNASRLFPSKEKPTMHSLRLVIESSPLSRAEKVAYVKSLSKCKTDQEVKAVMELVEEDIESLTN

SEQ ID NO: 4 - protein, 568 aa, synthetic construct
  REGION 1..568: note = Sendai virus P protein TS mutants
  SITE 433: note = MISC_FEATURE - X1 = any one of D, A, S, T, or G
  SITE 434: note = MISC_FEATURE - X2 = any one of R, A, S, T, or G
  SITE 437: note = MISC_FEATURE - X3 = any one of K, A, S, T, or G
  SITE 511: note = MISC_FEATURE - X3 = any one of L, F, or Y
MDQDAFILKEDSEVEREAPGGRESLSDVIGFLDAVLSSEPTDIGGDRSWLHNTINTPQGPGSAHRAKSEGEGEVSTPSTQDNRSGEESRVSGRTSKPEAEAHAGNLDKQNIHRAFGGRTGTNSVSQDLGDGGDSGILENPPNERGYPRSGIEDENREMAAHPDKRGEDQAEGLPEEVRGSTSLPDEGEGGASNNGRSMEPGSSHSARVTGVLVIPSPELEEAVLRRNKRRPTNSGSKPLTPATVPGTRSPPLNRYNSTGSPPGKPPSTQDEHINSGDTPAVRVKDRKPPIGTRSVSDCPANGRPIHPGLETDSTKKGIGENTSSMKEMATLLTSLGVIQSAQEFESSRDASYVFARRALKSANYAEMTFNVCGLILSAEKSSARKVDENKQLLKQIQESVESFRDIYKRFSEYQKEQNSLLMSNLSTLHIITXXGGXTDNTDSLTRSPSVFAKSKENKTKATRFDPSMETLEDMKYKPDLIREDEFRDEIRNPVYQERDTEPRASNASRLXPSKEKPTMHSLRLVIESSPLSRAEKVAYVKSLSKCKTDQEVKAVMELVEEDIESLTN

SEQ ID NO: 5 - protein, 2228 aa, Sendai virus
MDGQESSQNPSDILYPECHLNSPIVRGKIAQLHVLLDVNQPYRLKDDSIINITKHKIRNGGLSPRQIKIRSLGKALQRTIKDLDRYTFEPYPTYSQELLRLDIPEICDKIRSVFAVSDRLTRELSSGFQDLWLNIFKQLGNIEGREGYDPLQDIGTIPEITDKYSRNRWYRPFLTWFSIKYDMRWMQKTRPGGPLDTSNSHNLLECKSYTLVTYGDLVMILNKLTLTGYILTPELVLMYCDVVEGRWNMSAAGHLDKKSIGITSKGEELWELVDSLFSSLGEEIYNVIALLEPLSLALIQLNDPVIPLRGAFMRHVLTELQTVLTSRDVYTDAEADTIVESLLAIFHGTSIDEKAEIFSFFRTFGHPSLEAVTAADKVRAHMYAQKAIKLKTLYECHAVFCTIIINGYRERHGGQWPPCDFPDHVCLELRNAQGSNTAISYECAVDNYTSFIGFKFRKFIEPQLDEDLTIYMKDKALSPRKEAWDSVYPDSNLYYKAPESEETRRLIEVFINDENFNPEEIINYVESGDWLKDEEFNISYSLKEKEIKQEGRLFAKMTYKMRAVQVLAETLLAKGIGELFSENGMVKGEIDLLKRLTTLSVSGVPRTDSVYNNSKSSEKRNEGMENKNSGGYWDEKKRSRHEFKATDSSTDGYETLSCFLTTDLKKYCLNWRFESTALFGQRCNEIFGFKTFFNWMHPVLERCTIYVGDPYCPVADRMHRQLQDHADSGIFIHNPRGGIEGYCQKLWTLISISAIHLAAVRVGVRVSAMVQGDNQAIAVTSRVPVAQTYKQKKNHVYEEITKYFGALRHVMFDVGHELKLNETIISSKMFVYSKRIYYDGKILPQCLKALTKCVFWSETLVDENRSACSNISTSIAKAIENGYSPILGYCIALYKTCQQVCISLGMTINPTISPTVRDQYFKGKNWLRCAVLIPANVGGFNYMSTSRCFVRNIGDPAVAALADLKRFIRADLLDKQVLYRVMNQEPGDSSFLDWASDPYSCNLPHSQSITTIIKNITARSVLQESPNPLLSGLFTETSGEEDLNLASFLMDRKVILPRVAHEILGNSLTGVREAIAGMLDTTKSLVRASVRKGGLSYGILRRLVNYDLLQYETLTRTLRKPVKDNIEYEYMCSVELAVGLRQKMWIHLTYGRPIHGLETPDPLELLRGIFIEGSEVCKLCRSEGADPIYTWFYLPDNIDLDTLTNGCPAIRIPYFGSATDERSEAQLGYVRNLSKPAKAAIRIAMVYTWAYGTDEISWMEAALIAQTRANLSLENLKLLTPVSTSTNLSHRLKDTATQMKFSSATLVRASRFITISNDNMALKEAGESKDTNLVYQQIMLTGLSLFEFNMRYKKGSLGKPLILHLHLNNGCCIMESPQEANIPPRSTLDLEITQENNKLIYDPDPLKDVDLELFSKVRDVVHTVDMTYWSDDEVIRATSICTAMTIADTMSQLDRDNLKEMIALVNDDDVNSLITEFMVIDVPLFCSTFGGILVNQFAYSLYGLNIRGREEIWGHVVRILKDTSHAVLKVLSNALSHPKIFKRFWNAGVVEPVYGPNLSNQDKILLALSVCEYSVDLFMHDWQGGVPLEIFICDNDPDVADMRRSSFLARHLAYLCSLAEISRDGPRLESMNSLERLESLKSYLELTFLDDPVLRYSQLTGLVIKVFPSTLTYIRKSSIKVLRTRGIGVPEVLEDWDPEADNALLDGIAAEIQQNIPLGHQTRAPFWGLRVSKSQVLRLRGYKEITRGEIGRSGVGLTLPFDGRYLSHQLRLFGINSTSCLKALELTYLLSPLVDKDKDRLYLGEGAGAMLSCYDATLGPCINYYNSGVYSCDVNGQRELNIYPAEVALVGKKLNNVTSLGQRVKVLFNGNPGSTWIGNDECEALIWNELQNSSIGLVHCDMEGGDHKDDQVVLHEHYSVIRIAYLVGDRDVVLISKIAPRLGTDWTRQLSLYLRYWDEVNLIVLKTSNPASTEMYLLSRHPKSDIIEDSKTVLASLLPLSKEDSIKIEKWILIEKAKAHEWVTRELREGSSSSGMLRPYHQALQTFGFEPNLYKLSRDFLSTMNIADTHNCMIAFNRVLKDTIFEWARITESDKRLKLTGKYDLYPVRDSGKLKTISRRLVLSWISLSMSTRLVTGSFPDQKFEARLQLGIVSLSSREIRNLRVITKTLLDRFEDIIHSITYRFLTKEIKILMKILGAVKMFGARQNEYTTVIDDGSLGDIEPYDSS

SEQ ID NO: 6 - protein, 2228 aa, synthetic construct
  REGION 1..2228: note = Sendai virus L protein mutants
  SITE 1197: note = MISC_FEATURE - X1 = N or S
  SITE 1361: note = MISC_FEATURE - X2 = L or C
  SITE 1558: note = MISC_FEATURE - X3 = L or I
  SITE 1796: note = MISC_FEATURE - X4 = K or E
MDGQESSQNPSDILYPECHLNSPIVRGKIAQLHVLLDVNQPYRLKDDSIINITKHKIRNGGLSPRQIKIRSLGKALQRTIKDLDRYTFEPYPTYSQELLRLDIPEICDKIRSVFAVSDRLTRELSSGFQDLWLNIFKQLGNIEGREGYDPLQDIGTIPEITDKYSRNRWYRPFLTWFSIKYDMRWMQKTRPGGPLDTSNSHNLLECKSYTLVTYGDLVMILNKLTLTGYILTPELVLMYCDVVEGRWNMSAAGHLDKKSIGITSKGEELWELVDSLFSSLGEEIYNVIALLEPLSLALIQLNDPVIPLRGAFMRHVLTELQTVLTSRDVYTDAEADTIVESLLAIFHGTSIDEKAEIFSFFRTFGHPSLEAVTAADKVRAHMYAQKAIKLKTLYECHAVFCTIIINGYRERHGGQWPPCDFPDHVCLELRNAQGSNTAISYECAVDNYTSFIGFKFRKFIEPQLDEDLTIYMKDKALSPRKEAWDSVYPDSNLYYKAPESEETRRLIEVFINDENFNPEEIINYVESGDWLKDEEFNISYSLKEKEIKQEGRLFAKMTYKMRAVQVLAETLLAKGIGELFSENGMVKGEIDLLKRLTTLSVSGVPRTDSVYNNSKSSEKRNEGMENKNSGGYWDEKKRSRHEFKATDSSTDGYETLSCFLTTDLKKYCLNWRFESTALFGQRCNEIFGFKTFFNWMHPVLERCTIYVGDPYCPVADRMHRQLQDHADSGIFIHNPRGGIEGYCQKLWTLISISAIHLAAVRVGVRVSAMVQGDNQAIAVTSRVPVAQTYKQKKNHVYEEITKYFGALRHVMFDVGHELKLNETIISSKMFVYSKRIYYDGKILPQCLKALTKCVFWSETLVDENRSACSNISTSIAKAIENGYSPILGYCIALYKTCQQVCISLGMTINPTISPTVRDQYFKGKNWLRCAVLIPANVGGFNYMSTSRCFVRNIGDPAVAALADLKRFIRADLLDKQVLYRVMNQEPGDSSFLDWASDPYSCNLPHSQSITTIIKNITARSVLQESPNPLLSGLFTETSGEEDLNLASFLMDRKVILPRVAHEILGNSLTGVREAIAGMLDTTKSLVRASVRKGGLSYGILRRLVNYDLLQYETLTRTLRKPVKDNIEYEYMCSVELAVGLRQKMWIHLTYGRPIHGLETPDPLELLRGIFIEGSEVCKLCRSEGADPIYTWFYLPDXIDLDTLTNGCPAIRIPYFGSATDERSEAQLGYVRNLSKPAKAAIRIAMVYTWAYGTDEISWMEAALIAQTRANLSLENLKLLTPVSTSTNLSHRLKDTATQMKFSSATLVRASRFITISNDNMALKEAGESKDTNLVYQQIMLTGLSLFEFNMRYKKGSLGKPXILHLHLNNGCCIMESPQEANIPPRSTLDLEITQENNKLIYDPDPLKDVDLELFSKVRDVVHTVDMTYWSDDEVIRATSICTAMTIADTMSQLDRDNLKEMIALVNDDDVNSLITEFMVIDVPLFCSTFGGILVNQFAYSLYGLNIRGREEIWGHVVRILKDTSHAVLKVLSNALSHPKIFKRFWNAGVVEPVYGPNXSNQDKILLALSVCEYSVDLFMHDWQGGVPLEIFICDNDPDVADMRRSSFLARHLAYLCSLAEISRDGPRLESMNSLERLESLKSYLELTFLDDPVLRYSQLTGLVIKVFPSTLTYIRKSSIKVLRTRGIGVPEVLEDWDPEADNALLDGIAAEIQQNIPLGHQTRAPFWGLRVSKSQVLRLRGYKEITRGEIGRSGVGLTLPFDGRYLSHQLRLFGINSTSCLKALELTYLLSPLVDXDKDRLYLGEGAGAMLSCYDATLGPCINYYNSGVYSCDVNGQRELNIYPAEVALVGKKLNNVTSLGQRVKVLFNGNPGSTWIGNDECEALIWNELQNSSIGLVHCDMEGGDHKDDQVVLHEHYSVIRIAYLVGDRDVVLISKIAPRLGTDWTRQLSLYLRYWDEVNLIVLKTSNPASTEMYLLSRHPKSDIIEDSKTVLASLLPLSKEDSIKIEKWILIEKAKAHEWVTRELREGSSSSGMLRPYHQALQTFGFEPNLYKLSRDFLSTMNIADTHNCMIAFNRVLKDTIFEWARITESDKRLKLTGKYDLYPVRDSGKLKTISRRLVLSWISLSMSTRLVTGSFPDQKFEARLQLGIVSLSSREIRNLRVITKTLLDRFEDIIHSITYRFLTKEIKILMKILGAVKMFGARQNEYTTVIDDGSLGDIEPYDSS

SEQ ID NO: 7 - protein, 2228 aa, synthetic construct
  REGION 1..2228: note = Sendai virus L protein N1197S/L1558I/K1796E mutant
MDGQESSQNPSDILYPECHLNSPIVRGKIAQLHVLLDVNQPYRLKDDSIINITKHKIRNGGLSPRQIKIRSLGKALQRTIKDLDRYTFEPYPTYSQELLRLDIPEICDKIRSVFAVSDRLTRELSSGFQDLWLNIFKQLGNIEGREGYDPLQDIGTIPEITDKYSRNRWYRPFLTWFSIKYDMRWMQKTRPGGPLDTSNSHNLLECKSYTLVTYGDLVMILNKLTLTGYILTPELVLMYCDVVEGRWNMSAAGHLDKKSIGITSKGEELWELVDSLFSSLGEEIYNVIALLEPLSLALIQLNDPVIPLRGAFMRHVLTELQTVLTSRDVYTDAEADTIVESLLAIFHGTSIDEKAEIFSFFRTFGHPSLEAVTAADKVRAHMYAQKAIKLKTLYECHAVFCTIIINGYRERHGGQWPPCDFPDHVCLELRNAQGSNTAISYECAVDNYTSFIGFKFRKFIEPQLDEDLTIYMKDKALSPRKEAWDSVYPDSNLYYKAPESEETRRLIEVFINDENFNPEEIINYVESGDWLKDEEFNISYSLKEKEIKQEGRLFAKMTYKMRAVQVLAETLLAKGIGELFSENGMVKGEIDLLKRLTTLSVSGVPRTDSVYNNSKSSEKRNEGMENKNSGGYWDEKKRSRHEFKATDSSTDGYETLSCFLTTDLKKYCLNWRFESTALFGQRCNEIFGFKTFFNWMHPVLERCTIYVGDPYCPVADRMHRQLQDHADSGIFIHNPRGGIEGYCQKLWTLISISAIHLAAVRVGVRVSAMVQGDNQAIAVTSRVPVAQTYKQKKNHVYEEITKYFGALRHVMFDVGHELKLNETIISSKMFVYSKRIYYDGKILPQCLKALTKCVFWSETLVDENRSACSNISTSIAKAIENGYSPILGYCIALYKTCQQVCISLGMTINPTISPTVRDQYFKGKNWLRCAVLIPANVGGFNYMSTSRCFVRNIGDPAVAALADLKRFIRADLLDKQVLYRVMNQEPGDSSFLDWASDPYSCNLPHSQSITTIIKNITARSVLQESPNPLLSGLFTETSGEEDLNLASFLMDRKVILPRVAHEILGNSLTGVREAIAGMLDTTKSLVRASVRKGGLSYGILRRLVNYDLLQYETLTRTLRKPVKDNIEYEYMCSVELAVGLRQKMWIHLTYGRPIHGLETPDPLELLRGIFIEGSEVCKLCRSEGADPIYTWFYLPDSIDLDTLTNGCPAIRIPYFGSATDERSEAQLGYVRNLSKPAKAAIRIAMVYTWAYGTDEISWMEAALIAQTRANLSLENLKLLTPVSTSTNLSHRLKDTATQMKFSSATLVRASRFITISNDNMALKEAGESKDTNLVYQQIMLTGLSLFEFNMRYKKGSLGKPLILHLHLNNGCCIMESPQEANIPPRSTLDLEITQENNKLIYDPDPLKDVDLELFSKVRDVVHTVDMTYWSDDEVIRATSICTAMTIADTMSQLDRDNLKEMIALVNDDDVNSLITEFMVIDVPLFCSTFGGILVNQFAYSLYGLNIRGREEIWGHVVRILKDTSHAVLKVLSNALSHPKIFKRFWNAGVVEPVYGPNISNQDKILLALSVCEYSVDLFMHDWQGGVPLEIFICDNDPDVADMRRSSFLARHLAYLCSLAEISRDGPRLESMNSLERLESLKSYLELTFLDDPVLRYSQLTGLVIKVFPSTLTYIRKSSIKVLRTRGIGVPEVLEDWDPEADNALLDGIAAEIQQNIPLGHQTRAPFWGLRVSKSQVLRLRGYKEITRGEIGRSGVGLTLPFDGRYLSHQLRLFGINSTSCLKALELTYLLSPLVDEDKDRLYLGEGAGAMLSCYDATLGPCINYYNSGVYSCDVNGQRELNIYPAEVALVGKKLNNVTSLGQRVKVLFNGNPGSTWIGNDECEALIWNELQNSSIGLVHCDMEGGDHKDDQVVLHEHYSVIRIAYLVGDRDVVLISKIAPRLGTDWTRQLSLYLRYWDEVNLIVLKTSNPASTEMYLLSRHPKSDIIEDSKTVLASLLPLSKEDSIKIEKWILIEKAKAHEWVTRELREGSSSSGMLRPYHQALQTFGFEPNLYKLSRDFLSTMNIADTHNCMIAFNRVLKDTIFEWARITESDKRLKLTGKYDLYPVRDSGKLKTISRRLVLSWISLSMSTRLVTGSFPDQKFEARLQLGIVSLSSREIRNLRVITKTLLDRFEDIIHSITYRFLTKEIKILMKILGAVKMFGARQNEYTTVIDDGSLGDIEPYDSS

SEQ ID NO: 8 - protein, 568 aa, synthetic construct
  REGION 1..568: note = P2Y
MDQDAFILKEDSEVEREAPGGRESLSDVIGFLDAVLSSEPTDIGGDRSWLHNTINTPQGPGSAHRAKSEGEGEVSTPSTQDNRSGEESRVSGRTSKPEAEAHAGNLDKQNIHRAFGGRTGTNSVSQDLGDGGDSGILENPPNERGYPRSGIEDENREMAAHPDKRGEDQAEGLPEEVRGSTSLPDEGEGGASNNGRSMEPGSSHSARVTGVLVIPSPELEEAVLRRNKRRPTNSGSKPLTPATVPGTRSPPLNRYNSTGSPPGKPPSTQDEHINSGDTPAVRVKDRKPPIGTRSVSDCPANGRPIHPGLETDSTKKGIGENTSSMKEMATLLTSLGVIQSAQEFESSRDASYVFARRALKSANYAEMTFNVCGLILSAEKSSARKVDENKQLLKQIQESVESFRDIYKRFSEYQKEQNSLLMSNLSTLHIITAAGGATDNTDSLTRSPSVFAKSKENKTKATRFDPSMETLEDMKYKPDLIREDEFRDEIRNPVYQERDTEPRASNASRLYPSKEKPTMHSLRLVIESSPLSRAEKVAYVKSLSKCKTDQEVKAVMELVEEDIESLTN

SEQ ID NO: 9 - protein, 568 aa, synthetic construct
  REGION 1..568: note = P2m3SY
MDQDAFILKEDSEVEREAPGGRESLSDVIGFLDAVLSSEPTDIGGDRSWLHNTINTPQGPGSAHRAKSEGEGEVSTPSTQDNRSGEESRVSGRTSKPEAEAHAGNLDKQNIHRAFGGRTGTNSVSQDLGDGGDSGILENPPNERGYPRSGIEDENREMAAHPDKRGEDQAEGLPEEVRGSTSLPDEGEGGASNNGRSMEPGSSHSARVTGVLVIPSPELEEAVLRRNKRRPTNSGSKPLTPATVPGTRSPPLNRYNSTGSPPGKPPSTQDEHINSGDTPAVRVKDRKPPIGTRSVSDCPANGRPIHPGLETDSTKKGIGENTSSMKEMATLLTSLGVIQSAQEFESSRDASYVFARRALKSANYAEMTFNVCGLILSAEKSSARKVDENKQLLKQIQESVESFRDIYKRFSEYQKEQNSLLMSNLSTLHIITSSGGSTDNTDSLTRSPSVFAKSKENKTKATRFDPSMETLEDMKYKPDLIREDEFRDEIRNPVYQERDTEPRASNASRLYPSKEKPTMHSLRLVIESSPLSRAEKVAYVKSLSKCKTDQEVKAVMELVEEDIESLTN

SEQ ID NO: 10 - protein, 568 aa, synthetic construct
  REGION 1..568: note = P2m3TY
MDQDAFILKEDSEVEREAPGGRESLSDVIGFLDAVLSSEPTDIGGDRSWLHNTINTPQGPGSAHRAKSEGEGEVSTPSTQDNRSGEESRVSGRTSKPEAEAHAGNLDKQNIHRAFGGRTGTNSVSQDLGDGGDSGILENPPNERGYPRSGIEDENREMAAHPDKRGEDQAEGLPEEVRGSTSLPDEGEGGASNNGRSMEPGSSHSARVTGVLVIPSPELEEAVLRRNKRRPTNSGSKPLTPATVPGTRSPPLNRYNSTGSPPGKPPSTQDEHINSGDTPAVRVKDRKPPIGTRSVSDCPANGRPIHPGLETDSTKKGIGENTSSMKEMATLLTSLGVIQSAQEFESSRDASYVFARRALKSANYAEMTFNVCGLILSAEKSSARKVDENKQLLKQIQESVESFRDIYKRFSEYQKEQNSLLMSNLSTLHIITTTGGTTDNTDSLTRSPSVFAKSKENKTKATRFDPSMETLEDMKYKPDLIREDEFRDEIRNPVYQERDTEPRASNASRLYPSKEKPTMHSLRLVIESSPLSRAEKVAYVKSLSKCKTDQEVKAVMELVEEDIESLTN

SEQ ID NO: 11 - protein, 568 aa, synthetic construct
  REGION 1..568: note = P2m3GY
MDQDAFILKEDSEVEREAPGGRESLSDVIGFLDAVLSSEPTDIGGDRSWLHNTINTPQGPGSAHRAKSEGEGEVSTPSTQDNRSGEESRVSGRTSKPEAEAHAGNLDKQNIHRAFGGRTGTNSVSQDLGDGGDSGILENPPNERGYPRSGIEDENREMAAHPDKRGEDQAEGLPEEVRGSTSLPDEGEGGASNNGRSMEPGSSHSARVTGVLVIPSPELEEAVLRRNKRRPTNSGSKPLTPATVPGTRSPPLNRYNSTGSPPGKPPSTQDEHINSGDTPAVRVKDRKPPIGTRSVSDCPANGRPIHPGLETDSTKKGIGENTSSMKEMATLLTSLGVIQSAQEFESSRDASYVFARRALKSANYAEMTFNVCGLILSAEKSSARKVDENKQLLKQIQESVESFRDIYKRFSEYQKEQNSLLMSNLSTLHIITGGGGGTDNTDSLTRSPSVFAKSKENKTKATRFDPSMETLEDMKYKPDLIREDEFRDEIRNPVYQERDTEPRASNASRLYPSKEKPTMHSLRLVIESSPLSRAEKVAYVKSLSKCKTDQEVKAVMELVEEDIESLTN

SEQ ID NO: 12 - protein, 568 aa, synthetic construct
  REGION 1..568: note = P2m3SF
MDQDAFILKEDSEVEREAPGGRESLSDVIGFLDAVLSSEPTDIGGDRSWLHNTINTPQGPGSAHRAKSEGEGEVSTPSTQDNRSGEESRVSGRTSKPEAEAHAGNLDKQNIHRAFGGRTGTNSVSQDLGDGGDSGILENPPNERGYPRSGIEDENREMAAHPDKRGEDQAEGLPEEVRGSTSLPDEGEGGASNNGRSMEPGSSHSARVTGVLVIPSPELEEAVLRRNKRRPTNSGSKPLTPATVPGTRSPPLNRYNSTGSPPGKPPSTQDEHINSGDTPAVRVKDRKPPIGTRSVSDCPANGRPIHPGLETDSTKKGIGENTSSMKEMATLLTSLGVIQSAQEFESSRDASYVFARRALKSANYAEMTFNVCGLILSAEKSSARKVDENKQLLKQIQESVESFRDIYKRFSEYQKEQNSLLMSNLSTLHIITSSGGSTDNTDSLTRSPSVFAKSKENKTKATRFDPSMETLEDMKYKPDLIREDEFRDEIRNPVYQERDTEPRASNASRLFPSKEKPTMHSLRLVIESSPLSRAEKVAYVKSLSKCKTDQEVKAVMELVEEDIESLTN

SEQ ID NO: 13 - protein, 568 aa, synthetic construct
  REGION 1..568: note = P2m433S
MDQDAFILKEDSEVEREAPGGRESLSDVIGFLDAVLSSEPTDIGGDRSWLHNTINTPQGPGSAHRAKSEGEGEVSTPSTQDNRSGEESRVSGRTSKPEAEAHAGNLDKQNIHRAFGGRTGTNSVSQDLGDGGDSGILENPPNERGYPRSGIEDENREMAAHPDKRGEDQAEGLPEEVRGSTSLPDEGEGGASNNGRSMEPGSSHSARVTGVLVIPSPELEEAVLRRNKRRPTNSGSKPLTPATVPGTRSPPLNRYNSTGSPPGKPPSTQDEHINSGDTPAVRVKDRKPPIGTRSVSDCPANGRPIHPGLETDSTKKGIGENTSSMKEMATLLTSLGVIQSAQEFESSRDASYVFARRALKSANYAEMTFNVCGLILSAEKSSARKVDENKQLLKQIQESVESFRDIYKRFSEYQKEQNSLLMSNLSTLHIITSAGGATDNTDSLTRSPSVFAKSKENKTKATRFDPSMETLEDMKYKPDLIREDEFRDEIRNPVYQERDTEPRASNASRLFPSKEKPTMHSLRLVIESSPLSRAEKVAYVKSLSKCKTDQEVKAVMELVEEDIESLTN

SEQ ID NO: 14 - protein, 568 aa, synthetic construct
  REGION 1..568: note = P2m433SY
MDQDAFILKEDSEVEREAPGGRESLSDVIGFLDAVLSSEPTDIGGDRSWLHNTINTPQGPGSAHRAKSEGEGEVSTPSTQDNRSGEESRVSGRTSKPEAEAHAGNLDKQNIHRAFGGRTGTNSVSQDLGDGGDSGILENPPNERGYPRSGIEDENREMAAHPDKRGEDQAEGLPEEVRGSTSLPDEGEGGASNNGRSMEPGSSHSARVTGVLVIPSPELEEAVLRRNKRRPTNSGSKPLTPATVPGTRSPPLNRYNSTGSPPGKPPSTQDEHINSGDTPAVRVKDRKPPIGTRSVSDCPANGRPIHPGLETDSTKKGIGENTSSMKEMATLLTSLGVIQSAQEFESSRDASYVFARRALKSANYAEMTFNVCGLILSAEKSSARKVDENKQLLKQIQESVESFRDIYKRFSEYQKEQNSLLMSNLSTLHIITSAGGATDNTDSLTRSPSVFAKSKENKTKATRFDPSMETLEDMKYKPDLIREDEFRDEIRNPVYQERDTEPRASNASRLYPSKEKPTMHSLRLVIESSPLSRAEKVAYVKSLSKCKTDQEVKAVMELVEEDIESLTN

SEQ ID NO: 15 - protein, 568 aa, synthetic construct
  REGION 1..568: note = P2m434SY
MDQDAFILKEDSEVEREAPGGRESLSDVIGFLDAVLSSEPTDIGGDRSWLHNTINTPQGPGSAHRAKSEGEGEVSTPSTQDNRSGEESRVSGRTSKPEAEAHAGNLDKQNIHRAFGGRTGTNSVSQDLGDGGDSGILENPPNERGYPRSGIEDENREMAAHPDKRGEDQAEGLPEEVRGSTSLPDEGEGGASNNGRSMEPGSSHSARVTGVLVIPSPELEEAVLRRNKRRPTNSGSKPLTPATVPGTRSPPLNRYNSTGSPPGKPPSTQDEHINSGDTPAVRVKDRKPPIGTRSVSDCPANGRPIHPGLETDSTKKGIGENTSSMKEMATLLTSLGVIQSAQEFESSRDASYVFARRALKSANYAEMTFNVCGLILSAEKSSARKVDENKQLLKQIQESVESFRDIYKRFSEYQKEQNSLLMSNLSTLHIITASGGATDNTDSLTRSPSVFAKSKENKTKATRFDPSMETLEDMKYKPDLIREDEFRDEIRNPVYQERDTEPRASNASRLYPSKEKPTMHSLRLVIESSPLSRAEKVAYVKSLSKCKTDQEVKAVMELVEEDIESLTN

SEQ ID NO: 16 - protein, 568 aa, synthetic construct
  REGION 1..568: note = P2m437SY
MDQDAFILKEDSEVEREAPGGRESLSDVIGFLDAVLSSEPTDIGGDRSWLHNTINTPQGPGSAHRAKSEGEGEVSTPSTQDNRSGEESRVSGRTSKPEAEAHAGNLDKQNIHRAFGGRTGTNSVSQDLGDGGDSGILENPPNERGYPRSGIEDENREMAAHPDKRGEDQAEGLPEEVRGSTSLPDEGEGGASNNGRSMEPGSSHSARVTGVLVIPSPELEEAVLRRNKRRPTNSGSKPLTPATVPGTRSPPLNRYNSTGSPPGKPPSTQDEHINSGDTPAVRVKDRKPPIGTRSVSDCPANGRPIHPGLETDSTKKGIGENTSSMKEMATLLTSLGVIQSAQEFESSRDASYVFARRALKSANYAEMTFNVCGLILSAEKSSARKVDENKQLLKQIQESVESFRDIYKRFSEYQKEQNSLLMSNLSTLHIITAAGGSTDNTDSLTRSPSVFAKSKENKTKATRFDPSMETLEDMKYKPDLIREDEFRDEIRNPVYQERDTEPRASNASRLYPSKEKPTMHSLRLVIESSPLSRAEKVAYVKSLSKCKTDQEVKAVMELVEEDIESLTN

SEQ ID NO: 17 - protein, 2228 aa, synthetic construct
  REGION 1..2228: note = LmCI
MDGQESSQNPSDILYPECHLNSPIVRGKIAQLHVLLDVNQPYRLKDDSIINITKHKIRNGGLSPRQIKIRSLGKALQRTIKDLDRYTFEPYPTYSQELLRLDIPEICDKIRSVFAVSDRLTRELSSGFQDLWLNIFKQLGNIEGREGYDPLQDIGTIPEITDKYSRNRWYRPFLTWFSIKYDMRWMQKTRPGGPLDTSNSHNLLECKSYTLVTYGDLVMILNKLTLTGYILTPELVLMYCDVVEGRWNMSAAGHLDKKSIGITSKGEELWELVDSLFSSLGEEIYNVIALLEPLSLALIQLNDPVIPLRGAFMRHVLTELQTVLTSRDVYTDAEADTIVESLLAIFHGTSIDEKAEIFSFFRTFGHPSLEAVTAADKVRAHMYAQKAIKLKTLYECHAVFCTIIINGYRERHGGQWPPCDFPDHVCLELRNAQGSNTAISYECAVDNYTSFIGFKFRKFIEPQLDEDLTIYMKDKALSPRKEAWDSVYPDSNLYYKAPESEETRRLIEVFINDENFNPEEIINYVESGDWLKDEEFNISYSLKEKEIKQEGRLFAKMTYKMRAVQVLAETLLAKGIGELFSENGMVKGEIDLLKRLTTLSVSGVPRTDSVYNNSKSSEKRNEGMENKNSGGYWDEKKRSRHEFKATDSSTDGYETLSCFLTTDLKKYCLNWRFESTALFGQRCNEIFGFKTFFNWMHPVLERCTIYVGDPYCPVADRMHRQLQDHADSGIFIHNPRGGIEGYCQKLWTLISISAIHLAAVRVGVRVSAMVQGDNQAIAVTSRVPVAQTYKQKKNHVYEEITKYFGALRHVMFDVGHELKLNETIISSKMFVYSKRIYYDGKILPQCLKALTKCVFWSETLVDENRSACSNISTSIAKAIENGYSPILGYCIALYKTCQQVCISLGMTINPTISPTVRDQYFKGKNWLRCAVLIPANVGGFNYMSTSRCFVRNIGDPAVAALADLKRFIRADLLDKQVLYRVMNQEPGDSSFLDWASDPYSCNLPHSQSITTIIKNITARSVLQESPNPLLSGLFTETSGEEDLNLASFLMDRKVILPRVAHEILGNSLTGVREAIAGMLDTTKSLVRASVRKGGLSYGILRRLVNYDLLQYETLTRTLRKPVKDNIEYEYMCSVELAVGLRQKMWIHLTYGRPIHGLETPDPLELLRGIFIEGSEVCKLCRSEGADPIYTWFYLPDSIDLDTLTNGCPAIRIPYFGSATDERSEAQLGYVRNLSKPAKAAIRIAMVYTWAYGTDEISWMEAALIAQTRANLSLENLKLLTPVSTSTNLSHRLKDTATQMKFSSATLVRASRFITISNDNMALKEAGESKDTNLVYQQIMLTGLSLFEFNMRYKKGSLGKPCILHLHLNNGCCIMESPQEANIPPRSTLDLEITQENNKLIYDPDPLKDVDLELFSKVRDVVHTVDMTYWSDDEVIRATSICTAMTIADTMSQLDRDNLKEMIALVNDDDVNSLITEFMVIDVPLFCSTFGGILVNQFAYSLYGLNIRGREEIWGHVVRILKDTSHAVLKVLSNALSHPKIFKRFWNAGVVEPVYGPNISNQDKILLALSVCEYSVDLFMHDWQGGVPLEIFICDNDPDVADMRRSSFLARHLAYLCSLAEISRDGPRLESMNSLERLESLKSYLELTFLDDPVLRYSQLTGLVIKVFPSTLTYIRKSSIKVLRTRGIGVPEVLEDWDPEADNALLDGIAAEIQQNIPLGHQTRAPFWGLRVSKSQVLRLRGYKEITRGEIGRSGVGLTLPFDGRYLSHQLRLFGINSTSCLKALELTYLLSPLVDEDKDRLYLGEGAGAMLSCYDATLGPCINYYNSGVYSCDVNGQRELNIYPAEVALVGKKLNNVTSLGQRVKVLFNGNPGSTWIGNDECEALIWNELQNSSIGLVHCDMEGGDHKDDQVVLHEHYSVIRIAYLVGDRDVVLISKIAPRLGTDWTRQLSLYLRYWDEVNLIVLKTSNPASTEMYLLSRHPKSDIIEDSKTVLASLLPLSKEDSIKIEKWILIEKAKAHEWVTRELREGSSSSGMLRPYHQALQTFGFEPNLYKLSRDFLSTMNIADTHNCMIAFNRVLKDTIFEWARITESDKRLKLTGKYDLYPVRDSGKLKTISRRLVLSWISLSMSTRLVTGSFPDQKFEARLQLGIVSLSSREIRNLRVITKTLLDRFEDIIHSITYRFLTKEIKILMKILGAVKMFGARQNEYTTVIDDGSLGDIEPYDSS

SEQ ID NO: 18 - protein, 106 aa, synthetic construct
GVQVETISPGDGRTFPKRGQTCVVHYTGMLEDGKKVDSSRDRNKPFKFMLGKQEVIRGWEEGVAQMSVGQRAKLTISPDYAYGATGHPGIIPPHATLVFDVELLKP

SEQ ID NO: 19 - protein, 107 aa, synthetic construct
GVQIETISPGDGRTFPKKGQTCVVHYTGMLEDGKKLDSSRDRNKPFKFMIGKQEVIKGFEEGAAQMSLGQRAKLTISPDYAYGATGHPGVIPPHATLIFDVELLRPE

SEQ ID NO: 20 - protein, 348 aa, synthetic construct
MADIYRFPKFSYEDNGTVEPLPLRTGPDKKAIPHIRIVKVGDPPKHGVRYLDLLLLGFFETPKQTTNLESVSDLTEPTSYSICGSGSLPIGVAKYYGTDQELLKACTDLRITVRRAVRAGEMIVYMVDSIGAPLLPWSGRLRQGMIFNANKVALAPQCLPVDKDIRLRVVFVNGTSLGAITITKIPKTLADLALPNSISVNLLVTLKTGISTEQKGVLPVLDDQGEKKLNFMVHLGLIRRKVGKIYSVEYCKSKIERMRLIFSLGLIGGISFHVQVNGTLSKTFMSQLAWKRAVCFPLMDVNPHMNMVIWAASVEITGVDAVFQPAIPRDFRYYPNVVAKNIGRIRKL

SEQ ID NO: 21 - protein, 575 aa, synthetic construct
MDGDRGKRDSYWSTSPSGSTTKPASGWERSSKADTWLLILSFTQWALSIATVIICIIISARQGYSMKEYSMTVEALNMSSREVKESLTSLIRQEVIARAVNIQSSVQTGIPVLLNKNSRDVIQMIDKSCSRQELTQHCESTIAVHHADGIAPLEPHSFWRCPVGEPYLSSDPEISLLPGPSLLSGSTTISGCVRLPSLSIGEAIYAYSSNLITQGCADIGKSYQVLQLGYISLNSDMFPDLNPVVSHTYDINDNRKSCSVVTTKTRGYQLCSMPTVDERTDYSSDGIEDLVLDVLDLKGRTKSHRYRNSEVDLDHPFSALYPSVGNGIATEGSLIFLGYGGLTTPLQGDTKCRTQGCQQVSQDTCNEALKITWLGGKQVVSVIIQVNDYLSERPKIRVTTIPITQNYLGAEGRLLKLGDRVYIYTRSSGWHSQLQIGVLDVSHPLTINWTPHEALSRPGNEECNWYNKCPKECISGVYTDAYPLSPDAANVATVTLYANTSRVNPTIMYSNTTNIINMLRIKDVQLEAAYTTTSCITHFGKGYCFHIIEINQKSLNTLQPMLFKTSIPKLCKAES

SEQ ID NO: 22 - protein, 108 aa, Bos taurus
MGVQVETISPGDGRTFPKRGQTCVVHYTGMLEDGKKFDSSRDRNKPFKFVLGKQEVIRGWEEGVAQMSVGQRAKLTISPDYAYGATGHPGIIPPNATLIFDVELLKLE

SEQ ID NO: 23 - protein, 108 aa, Macaca mulatta
MGVEIETISPGDGRTFPKKGQTCVVHYTGMLQNGKKFDSSRDRNKPFKFRIGKQEVIKGFEEGAAQMSLGQRAKLTCTPDVAYGATGHPGVIPPNATLIFDVELLNLE

SEQ ID NO: 24 - protein, 108 aa, Homo sp.
MGVQVETISPGDGRTFPKRGQTCVVHYTGMLEDGKKFDSSRDRNKPFKFMLGKQEVIRGWEEGVAQMSVGQRAKLTISPDYAYGATGHPGIIPPHATLVFDVELLKLE

SEQ ID NO: 25 - protein, 108 aa, Mus musculus
MGVEIETISPGDGRTFPKKGQICVVHYTGMLQNGKKFDSSRDRNKPFKFRIGKQEVIKGFEEGTAQMSLGQRAKLTCTPDVAYGATGHPGVIPPNATLIFDVELLSLE

SEQ ID NO: 26 - protein, 108 aa, Oryctolagus cuniculus; identical to SEQ ID NO: 24

SEQ ID NO: 27 - protein, 108 aa, Rattus norvegicus
MGVEIETISPGDGRTFPKKGQICVVHYTGMLQNGKKFDSSRDRNKPFKFRIGKQEVIKGFEEGAAQMSLGQRAKLTCTPDVAYGATGHPGVIPPNATLIFDVELLNLE

SEQ ID NO: 28 - protein, 107 aa, synthetic construct
GVQVETISPGDGRTFPRRGQTCVVHYTGMLEDGRRVDSSRDRNRPFRFMLGRQEVIRGWEEGVSQMSVGQRSRLTISPDYSYGSTGHPGIIPPHSTLVFDVELLRPE

SEQ ID NO: 29 - protein, 129 aa, synthetic construct
VKDVPDSQQHPAPEKSSKVSEQLKCCSGILKEMFAKKHAAYAWPFYKPVDVEALGAHDYCDIIKHPMDMSTIKSKLEAREYRDAQEFGADVRLMFSNCYKYNPPDHEVVAMARKLQDVFEMRFAKMPDE

SEQ ID NO: 30 - protein, 703 aa, synthetic construct
MDQDAFILKEDSEVEREAPGGRESLSDVIGFLDAVLSSEPTDIGGDRSWLHNTINTPQGPGSAHRAKSEGEGEVSTPSTQDNRSGEESRVSGRTSKPEAEAHAGNLDKQNIHRAFGGRTGTNSVSQDLGDGGDSGILENPPNERGYPRSGIEDENREMAAHPDKRGEDQAEGLPEEVRGSTSLPDEGEGGASNNGRSMEPGSSHSARVTGVLVIPSPELEEAVLRRNKRRPTNSGSKPLTPATVPGTRSPPLNRYNSTGSPPGKPPSTQDEHINSGDTPAVRVKDRKPPIGTRSVSDCPANGRPIHPGLETDSTKKGIGENTSSMKEMATLLTSLGVIQSAQEFESSRDASYVFARRALKSANYAEMTFNVCGLILSAEKSSARKVDENKQLLKQIQESVESFRDIYKRFSEYQKEQNSLLMSNLSTLHIITSSGGSTDNTDSLTRSPSVFAKSKENKTKATRFDPSMETLEDMKYKPDLIREDEFRDEIRNPVYQERDTEPRASNASRLYPSKEKPTMHSLRLVIESSPLSRAEKVAYVKSLSKCKTDQEVKAVMELVEEDIESLTNKLGSGSVKDVPDSQQHPAPEKSSKVSEQLKCCSGILKEMFAKKHAAYAWPFYKPVDVEALGAHDYCDIIKHPMDMSTIKSKLEAREYRDAQEFGADVRLMFSNCYKYNPPDHEVVAMARKLQDVFEMRFAKMPDE

SEQ ID NO: 31 - protein, 703 aa, synthetic construct
MDQDAFILKEDSEVEREAPGGRESLSDVIGFLDAVLSSEPTDIGGDRSWLHNTINTPQGPGSAHRAKSEGEGEVSTPSTQDNRSGEESRVSGRTSKPEAEAHAGNLDKQNIHRAFGGRTGTNSVSQDLGDGGDSGILENPPNERGYPRSGIEDENREMAAHPDKRGEDQAEGLPEEVRGSTSLPDEGEGGASNNGRSMEPGSSHSARVTGVLVIPSPELEEAVLRRNKRRPTNSGSKPLTPATVPGTRSPPLNRYNSTGSPPGKPPSTQDEHINSGDTPAVRVKDRKPPIGTRSVSDCPANGRPIHPGLETDSTKKGIGENTSSMKEMATLLTSLGVIQSAQEFESSRDASYVFARRALKSANYAEMTFNVCGLILSAEKSSARKVDENKQLLKQIQESVESFRDIYKRFSEYQKEQNSLLMSNLSTLHIITSTGGSTDNTDSLTRSPSVFAKSKENKTKATRFDPSMETLEDMKYKPDLIREDEFRDEIRNPVYQERDTEPRASNASRLYPSKEKPTMHSLRLVIESSPLSRAEKVAYVKSLSKCKTDQEVKAVMELVEEDIESLTNKLGSGSVKDVPDSQQHPAPEKSSKVSEQLKCCSGILKEMFAKKHAAYAWPFYKPVDVEALGAHDYCDIIKHPMDMSTIKSKLEAREYRDAQEFGADVRLMFSNCYKYNPPDHEVVAMARKLQDVFEMRFAKMPDE

SEQ ID NO: 32 - protein, 703 aa, synthetic construct
MDQDAFILKEDSEVEREAPGGRESLSDVIGFLDAVLSSEPTDIGGDRSWLHNTINTPQGPGSAHRAKSEGEGEVSTPSTQDNRSGEESRVSGRTSKPEAEAHAGNLDKQNIHRAFGGRTGTNSVSQDLGDGGDSGILENPPNERGYPRSGIEDENREMAAHPDKRGEDQAEGLPEEVRGSTSLPDEGEGGASNNGRSMEPGSSHSARVTGVLVIPSPELEEAVLRRNKRRPTNSGSKPLTPATVPGTRSPPLNRYNSTGSPPGKPPSTQDEHINSGDTPAVRVKDRKPPIGTRSVSDCPANGRPIHPGLETDSTKKGIGENTSSMKEMATLLTSLGVIQSAQEFESSRDASYVFARRALKSANYAEMTFNVCGLILSAEKSSARKVDENKQLLKQIQESVESFRDIYKRFSEYQKEQNSLLMSNLSTLHIITTTGGTTDNTDSLTRSPSVFAKSKENKTKATRFDPSMETLEDMKYKPDLIREDEFRDEIRNPVYQERDTEPRASNASRLYPSKEKPTMHSLRLVIESSPLSRAEKVAYVKSLSKCKTDQEVKAVMELVEEDIESLTNKLGSGSVKDVPDSQQHPAPEKSSKVSEQLKCCSGILKEMFAKKHAAYAWPFYKPVDVEALGAHDYCDIIKHPMDMSTIKSKLEAREYRDAQEFGADVRLMFSNCYKYNPPDHEVVAMARKLQDVFEMRFAKMPDE

SEQ ID NO: 33 - protein, 373 aa, synthetic construct
MVSKGEELFTGVVPILVELDGDVNGHKFSVSGEGEGDATYGKLTLKFICTTGKLPVPWPTLVTTLTYGVQCFARYPDHMKQHDFFKSAMPEGYVQERTIFFKDDGNYKTRAEVKFEGDTLVNRIELKGIDFKEDGNILGHKLEYNYNSHKVYITADKQKNGIKVNFKTRHNIEDGSVQLADHYQQNTPIGDGPVLLPDNHYLSTQSALSKDPNEKRDHMVLLEFVTAAGITLGMDELYKLGSGSVKDVPDSQQHPAPEKSSKVSEQLKCCSGILKEMFAKKHAAYAWPFYKPVDVEALGAHDYCDIIKHPMDMSTIKSKLEAREYRDAQEFGADVRLMFSNCYKYNPPDHEVVAMARKLQDVFEMRFAKMPDE